European Patent Specification EP 2 283 851 B1, published June 7, 2023. Title: COMPOSITIONS AND METHODS FOR PROMOTING HEMOSTASIS AND OTHER PHYSIOLOGICAL ACTIVITIES. Applicant: Massachusetts Institute of Technology. Application PCT/US2006/015850. The sequence listing filed with the application follows.

SEQUENCE LISTING (76 sequences)

SEQ ID NO: 1 - protein, 16 aa, Artificial Sequence
  Synthetically generated peptide
RADARADARADARADA

SEQ ID NO: 2 - protein, 12 aa, Artificial Sequence
  Synthetically generated peptide
RADRDARADRDA

SEQ ID NO: 3 - protein, 8 aa, Artificial Sequence
  Synthetically generated peptide
RADARADA

SEQ ID NO: 4 - protein, 16 aa, Artificial Sequence
  Synthetically generated peptide
RARADADARARADADA

SEQ ID NO: 5 - protein, 8 aa, Artificial Sequence
  Synthetically generated peptide
RARADADA

SEQ ID NO: 6 - protein, 16 aa, Artificial Sequence
  Synthetically generated peptide
AEAKAEAKAEAKAEAK

SEQ ID NO: 7 - protein, 8 aa, Artificial Sequence
  Synthetically generated peptide
AEAKAEAK

SEQ ID NO: 8 - protein, 16 aa, Artificial Sequence
  Synthetically generated peptide
RAEARAEARAEARAEA

SEQ ID NO: 9 - protein, 8 aa, Artificial Sequence
  Synthetically generated peptide
RAEARAEA

SEQ ID NO: 10 - protein, 16 aa, Artificial Sequence
  Synthetically generated peptide
KADAKADAKADAKADA

SEQ ID NO: 11 - protein, 8 aa, Artificial Sequence
  Synthetically generated peptide
KADAKADA

SEQ ID NO: 12 - protein, 16 aa, Artificial Sequence
  Synthetically generated peptide
AEAEAHAHAEAEAHAH

SEQ ID NO: 13 - protein, 8 aa, Artificial Sequence
  Synthetically generated peptide
AEAEAHAH

SEQ ID NO: 14 - protein, 16 aa, Artificial Sequence
  Synthetically generated peptide
FEFEFKFKFEFEFKFK

SEQ ID NO: 15 - protein, 8 aa, Artificial Sequence
  Synthetically generated peptide
FEFKFEFK

SEQ ID NO: 16 - protein, 16 aa, Artificial Sequence
  Synthetically generated peptide
LELELKLKLELELKLK

SEQ ID NO: 17 - protein, 8 aa, Artificial Sequence
  Synthetically generated peptide
LELELKLK

SEQ ID NO: 18 - protein, 16 aa, Artificial Sequence
  Synthetically generated peptide
AEAEAKAKAEAEAKAK

SEQ ID NO: 19 - protein, 12 aa, Artificial Sequence
  Synthetically generated peptide
AEAEAEAEAKAK

SEQ ID NO: 20 - protein, 8 aa, Artificial Sequence
  Synthetically generated peptide
AEAEAKAK

SEQ ID NO: 21 - protein, 16 aa, Artificial Sequence
  Synthetically generated peptide
KAKAKAKAEAEAEAEA

SEQ ID NO: 22 - protein, 16 aa, Artificial Sequence
  Synthetically generated peptide
AEAEAEAEAKAKAKAK

SEQ ID NO: 23 - protein, 16 aa, Artificial Sequence
  Synthetically generated peptide
RARARARADADADADA

SEQ ID NO: 24 - protein, 16 aa, Artificial Sequence
  Synthetically generated peptide
ADADADADARARARAR

SEQ ID NO: 25 - protein, 16 aa, Artificial Sequence
  Synthetically generated peptide
DADADADARARARARA

SEQ ID NO: 26 - protein, 16 aa, Artificial Sequence
  Synthetically generated peptide
ADADADADARARARAR

SEQ ID NO: 27 - protein, 16 aa, Artificial Sequence
  Synthetically generated peptide
HEHEHKHKHEHEHKHK

SEQ ID NO: 28 - protein, 8 aa, Artificial Sequence
  Synthetically generated peptide
HEHEHKHK

SEQ ID NO: 29 - protein, 20 aa, Artificial Sequence
  Synthetically generated peptide
VEVEVEVEVEVEVEVEVEVE

SEQ ID NO: 30 - protein, 20 aa, Artificial Sequence
  Synthetically generated peptide
RFRFRFRFRFRFRFRFRFRF

SEQ ID NO: 31 - protein, 12 aa, Artificial Sequence
  Synthetically generated peptide
RADARADARADA

SEQ ID NO: 32 - protein, 16 aa, Artificial Sequence
  Synthetically generated peptide
AKAKAEAEAKAKAEAE

SEQ ID NO: 33 - protein, 16 aa, Artificial Sequence
  Synthetically generated peptide
AKAEAKAEAKAEAKAE

SEQ ID NO: 34 - protein, 16 aa, Artificial Sequence
  Synthetically generated peptide
EAKAEAKAEAKAEAKA

SEQ ID NO: 35 - protein, 16 aa, Artificial Sequence
  Synthetically generated peptide
KAEAKAEAKAEAKAEA

SEQ ID NO: 36 - protein, 16 aa, Artificial Sequence
  Synthetically generated peptide
ADADARARADADARAR

SEQ ID NO: 37 - protein, 16 aa, Artificial Sequence
  Synthetically generated peptide
ARADARADARADARAD

SEQ ID NO: 38 - protein, 16 aa, Artificial Sequence
  Synthetically generated peptide
DARADARADARADARA

SEQ ID NO: 39 - protein, 16 aa, Artificial Sequence
  Synthetically generated peptide
ADARADARADARADAR

SEQ ID NO: 40 - protein, 16 aa, Artificial Sequence
  Synthetically generated peptide
ARADAKAEARADAKAE

SEQ ID NO: 41 - protein, 16 aa, Artificial Sequence
  Synthetically generated peptide
AKAEARADAKAEARAD

SEQ ID NO: 42 - protein, 16 aa, Artificial Sequence
  Synthetically generated peptide
ARAKADAEARAKADAE

SEQ ID NO: 43 - protein, 16 aa, Artificial Sequence
  Synthetically generated peptide
AKARAEADAKARADAE

SEQ ID NO: 44 - protein, 16 aa, Artificial Sequence
  Synthetically generated peptide
AQAQAQAQAQAQAQAQ

SEQ ID NO: 45 - protein, 16 aa, Artificial Sequence
  Synthetically generated peptide
VQVQVQVQVQVQVQVQ

SEQ ID NO: 46 - protein, 16 aa, Artificial Sequence
  Synthetically generated peptide
YQYQYQYQYQYQYQYQ

SEQ ID NO: 47 - protein, 16 aa, Artificial Sequence
  Synthetically generated peptide
HQHQHQHQHQHQHQHQ

SEQ ID NO: 48 - protein, 15 aa, Artificial Sequence
  Synthetically generated peptide
ANANANANANANANA

SEQ ID NO: 49 - protein, 15 aa, Artificial Sequence
  Synthetically generated peptide
VNVNVNVNVNVNVNV

SEQ ID NO: 50 - protein, 15 aa, Artificial Sequence
  Synthetically generated peptide
YNYNYNYNYNYNYNY

SEQ ID NO: 51 - protein, 15 aa, Artificial Sequence
  Synthetically generated peptide
HNHNHNHNHNHNHNH

SEQ ID NO: 52 - protein, 16 aa, Artificial Sequence
  Synthetically generated peptide
ANAQANAQANAQANAQ

SEQ ID NO: 53 - protein, 15 aa, Artificial Sequence
  Synthetically generated peptide
AQANAQANAQANAQA

SEQ ID NO: 54 - protein, 16 aa, Artificial Sequence
  Synthetically generated peptide
VNVQVNVQVNVQVNVQ

SEQ ID NO: 55 - protein, 15 aa, Artificial Sequence
  Synthetically generated peptide
VQVNVQVNVQVNVQV

SEQ ID NO: 56 - protein, 16 aa, Artificial Sequence
  Synthetically generated peptide
YNYQYNYQYNYQYNYQ

SEQ ID NO: 57 - protein, 15 aa, Artificial Sequence
  Synthetically generated peptide
YQYNYQYNYQYNYQY

SEQ ID NO: 58 - protein, 16 aa, Artificial Sequence
  Synthetically generated peptide
HNHQHNHQHNHQHNHQ

SEQ ID NO: 59 - protein, 15 aa, Artificial Sequence
  Synthetically generated peptide
HQHNHQHNHQHNHQH

SEQ ID NO: 60 - protein, 18 aa, Artificial Sequence
  Synthetically generated peptide
AKAQADAKAQADAKAQAD

SEQ ID NO: 61 - protein, 18 aa, Artificial Sequence
  Synthetically generated peptide
VKVQVDVKVQVDVKVQVD

SEQ ID NO: 62 - protein, 18 aa, Artificial Sequence
  Synthetically generated peptide
YKYQYDYKYQYDYKYQYD

SEQ ID NO: 63 - protein, 18 aa, Artificial Sequence
  Synthetically generated peptide
HKHQHDHKHQHDHKHQHD

SEQ ID NO: 64 - protein, 16 aa, Artificial Sequence
  Synthetically generated peptide
ADADAKAKADADAKAK

SEQ ID NO: 65 - protein, 16 aa, Artificial Sequence
  Synthetically generated peptide
KAKAKAKAKAKAKAKA

SEQ ID NO: 66 - protein, 16 aa, Artificial Sequence
  Synthetically generated peptide
EAEAEAEAEAEAEAEA

SEQ ID NO: 67 - protein, 16 aa, Artificial Sequence
  Synthetically generated peptide
ADADADADADADADAD

SEQ ID NO: 68 - protein, 16 aa, Artificial Sequence
  Synthetically generated peptide
ARARADADARARADAD

SEQ ID NO: 69 - protein, 16 aa, Artificial Sequence
  Synthetically generated peptide
VRVRVDVDVRVRVDVD

SEQ ID NO: 70 - protein, 12 aa, Artificial Sequence
  Synthetically generated peptide
ARADARADARAD

SEQ ID NO: 71 - protein, 12 aa, Artificial Sequence
  Synthetically generated peptide
AKADAKADAKAD

SEQ ID NO: 72 - protein, 12 aa, Artificial Sequence
  Synthetically generated peptide
AHADAHADAHAD

SEQ ID NO: 73 - protein, 12 aa, Artificial Sequence
  Synthetically generated peptide
ARAEARAEARAE

SEQ ID NO: 74 - protein, 12 aa, Artificial Sequence
  Synthetically generated peptide
AKAEAKAEAKAE

SEQ ID NO: 75 - protein, 12 aa, Artificial Sequence
  Synthetically generated peptide
AHAEAHAEAHAE

SEQ ID NO: 76 - protein, 12 aa, Artificial Sequence
  Synthetically generated peptide
RARARADADADA